European Patent Specification EP 3 998 351 B1, published September 2, 2026. Title: PRIMERS WITH SELF-COMPLEMENTARY SEQUENCES FOR MULTIPLE DISPLACEMENT AMPLIFICATION. Applicant: Qiagen Sciences, LLC. Application New Divisional application based on EP17714992.9. The sequence listing filed with the application follows.

SEQUENCE LISTING (8 sequences)

SEQ ID NO: 1 - DNA, 12 bp, Artificial Sequence
  Primer sequence
cgatcatgatcg

SEQ ID NO: 2 - DNA, 18 bp, Artificial Sequence
  Primer sequence
cgatcacggccgtgatcg

SEQ ID NO: 3 - DNA, 12 bp, Artificial Sequence
  Primer sequence
  misc_feature (1)...(12): n = A,T,C or G
tgatcgnnnnnn

SEQ ID NO: 4 - DNA, 16 bp, Artificial Sequence
  Primer sequence
  misc_feature (1)...(16): n = A,T,C or G
gccgtgatcgnnnnnn

SEQ ID NO: 5 - DNA, 24 bp, Artificial Sequence
  Primer sequence
  misc_feature (1)...(24): n = A,T,C or G
cgatcacggccgtgatcgnnnnnn

SEQ ID NO: 6 - DNA, 18 bp, Artificial Sequence
  Primer sequence
  misc_feature (1)...(18): n = A,T,C or G
cgatcatgatcgnnnnnn

SEQ ID NO: 7 - DNA, 16 bp, Artificial Sequence
  Primer sequence
  misc_feature (1)...(16): n = A,T,C or G
cgatcgatcgnnnnnn

SEQ ID NO: 8 - DNA, 14 bp, Artificial Sequence
  Primer sequence
  misc_feature (1)...(14): n = A,T,C or G
cgatatcgnnnnnn